European Patent Specification EP 4 022 088 B1, published September 17, 2025. Title: COMPISITIONS AND METHODS OF TREATING AND REDUCING RISK OF CONDITIONS ASSOCIATED WITH ELEVATED 4-ETHYLPHENYL SULFATE IN CANINES AND IDENTIFTYING CANINES AT RISK OF SUCH CONDITIONS. Applicant: Hill's Pet Nutrition, Inc. The sequence listing filed with the application follows.

SEQUENCE LISTING (1 sequence)

SEQ ID NO: 1 - DNA, 201 bp, Canis familiaris
tatttgtcttgaaatttcattataagcttaatttttccttgttgttggtatcagactaccgtgtatgcttgttttctgtttccctccacggcaatctaccraaataaaatgaggtgtggttcctttgtcctttctgtaactctcagtcctcccccccaccccatatcctttacttgaggagggagactacatctaatttgg